European Patent Application EP 4 644 533 A1, published November 5, 2025. Title: CONSTRUCTION AND USE OF ENGINEERING BACTERIUM THAT PRODUCES COLANIC ACID WITH HIGH YIELD. Applicant: Shenzhen PAM2L Biotechnologies Co., Ltd. The sequence listing filed with the application follows.

SEQUENCE LISTING (75 sequences)

SEQ ID NO: 1 - DNA, 68 bp, synthetic construct
  source 1..68: mol_type = other DNA
ttgacaattaatcatcggctcgtataatgtgatcagacctttgtttaactttaagaaggagatatacc

SEQ ID NO: 2 - DNA, 35 bp, synthetic construct
  source 1..35: mol_type = other DNA
ttgacagctagctcagtcctaggtataatactagt

SEQ ID NO: 3 - DNA, 19 bp, synthetic construct
  source 1..19: mol_type = other DNA
taatacgactcactatagg

SEQ ID NO: 4 - DNA, 30 bp, synthetic construct
  source 1..30: mol_type = other DNA
gtttatacataggcgagtactctgttatgg

SEQ ID NO: 5 - DNA, 10 bp, synthetic construct
  source 1..10: mol_type = other DNA
aagaagggga

SEQ ID NO: 6 - DNA, 10 bp, synthetic construct
  source 1..10: mol_type = other DNA
aagaagagga

SEQ ID NO: 7 - DNA, 10 bp, synthetic construct
  source 1..10: mol_type = other DNA
aagaaggggc

SEQ ID NO: 8 - DNA, 10 bp, synthetic construct
  source 1..10: mol_type = other DNA
aagaggggga

SEQ ID NO: 9 - DNA, 10 bp, synthetic construct
  source 1..10: mol_type = other DNA
ggaaagggga

SEQ ID NO: 10 - DNA, 10 bp, synthetic construct
  source 1..10: mol_type = other DNA
agagagggga

SEQ ID NO: 11 - DNA, 10 bp, synthetic construct
  source 1..10: mol_type = other DNA
aagaagggag

SEQ ID NO: 12 - DNA, 10 bp, synthetic construct
  source 1..10: mol_type = other DNA
aggtagggga

SEQ ID NO: 13 - DNA, 10 bp, synthetic construct
  source 1..10: mol_type = other DNA
aagagaggag

SEQ ID NO: 14 - DNA, 10 bp, synthetic construct
  source 1..10: mol_type = other DNA
aggtaggggc

SEQ ID NO: 15 - DNA, 10 bp, synthetic construct
  source 1..10: mol_type = other DNA
aggtaggtga

SEQ ID NO: 16 - DNA, 10 bp, synthetic construct
  source 1..10: mol_type = other DNA
aggtagtgga

SEQ ID NO: 17 - DNA, 10 bp, synthetic construct
  source 1..10: mol_type = other DNA
aggtagcgga

SEQ ID NO: 18 - DNA, 10 bp, synthetic construct
  source 1..10: mol_type = other DNA
aggcgaggga

SEQ ID NO: 19 - DNA, 10 bp, synthetic construct
  source 1..10: mol_type = other DNA
aggacaggga

SEQ ID NO: 20 - DNA, 10 bp, synthetic construct
  source 1..10: mol_type = other DNA
aggtaggggt

SEQ ID NO: 21 - DNA, 10 bp, synthetic construct
  source 1..10: mol_type = other DNA
cggtagggga

SEQ ID NO: 22 - DNA, 10 bp, synthetic construct
  source 1..10: mol_type = other DNA
atagagggga

SEQ ID NO: 23 - DNA, 10 bp, synthetic construct
  source 1..10: mol_type = other DNA
aaagattaga

SEQ ID NO: 24 - DNA, 10 bp, synthetic construct
  source 1..10: mol_type = other DNA
aaagatatca

SEQ ID NO: 25 - DNA, 10 bp, synthetic construct
  source 1..10: mol_type = other DNA
aagagtagta

SEQ ID NO: 26 - DNA, 10 bp, synthetic construct
  source 1..10: mol_type = other DNA
aaaagggata

SEQ ID NO: 27 - DNA, 10 bp, synthetic construct
  source 1..10: mol_type = other DNA
agagagaata

SEQ ID NO: 28 - DNA, 10 bp, synthetic construct
  source 1..10: mol_type = other DNA
gagaggcaga

SEQ ID NO: 29 - DNA, 10 bp, synthetic construct
  source 1..10: mol_type = other DNA
gagacaagga

SEQ ID NO: 30 - DNA, 10 bp, synthetic construct
  source 1..10: mol_type = other DNA
gggaaagaga

SEQ ID NO: 31 - DNA, 10 bp, synthetic construct
  source 1..10: mol_type = other DNA
gaggacggag

SEQ ID NO: 32 - RNA, 31 nt, synthetic construct
  source 1..31: mol_type = other RNA
atgaatatgttcgtcaaatcctgcctgaagc

SEQ ID NO: 33 - RNA, 51 nt, synthetic construct
  source 1..51: mol_type = other RNA
gttttaacgatcaaaacccgcatccggcagagctcttatgcgtcgcgattc

SEQ ID NO: 34 - RNA, 54 nt, synthetic construct
  source 1..54: mol_type = other RNA
gaatcgcgacgcataagagctctgccggatgcgggttttgatcgttaaaacatc

SEQ ID NO: 35 - RNA, 26 nt, synthetic construct
  source 1..26: mol_type = other RNA
gcgatagcataatcgccctgggtttg

SEQ ID NO: 36 - RNA, 27 nt, synthetic construct
  source 1..27: mol_type = other RNA
cgcgctattgttacaagaggaagcctg

SEQ ID NO: 37 - RNA, 71 nt, synthetic construct
  source 1..71: mol_type = other RNA
cttcagctgacaggaatgcacaattgttttacctttataatgatgataacttttccaaaactgcttgactg

SEQ ID NO: 38 - RNA, 52 nt, synthetic construct
  source 1..52: mol_type = other RNA
gttatcatcattataaaggtaaaacaattgtgcattcctgtcagctgaaggg

SEQ ID NO: 39 - RNA, 33 nt, synthetic construct
  source 1..33: mol_type = other RNA
ctcctgtcatcagtacgctcaagcagaattatc

SEQ ID NO: 40 - RNA, 71 nt, synthetic construct
  source 1..71: mol_type = other RNA
atttcgaaaaatcctggtcataaaggttttacctttataatgatgataacttttccaaaactgcttgactg

SEQ ID NO: 41 - RNA, 61 nt, synthetic construct
  source 1..61: mol_type = other RNA
gttatcatcattataaaggtaaaacctttatgaccaggatttttcgaaatggcttttccac

SEQ ID NO: 42 - RNA, 27 nt, synthetic construct
  source 1..27: mol_type = other RNA
cttcttcattttgcgcagcaatcagcg

SEQ ID NO: 43 - RNA, 33 nt, synthetic construct
  source 1..33: mol_type = other RNA
ctatcattacaactgcctcgcttgttataagcg

SEQ ID NO: 44 - RNA, 51 nt, synthetic construct
  source 1..51: mol_type = other RNA
accttgctcatccattgcttcttccagcgtttcaagtgtacattctcttgc

SEQ ID NO: 45 - RNA, 49 nt, synthetic construct
  source 1..49: mol_type = other RNA
tacacttgaaacgctggaagaagcaatggatgagcaaggtaaatccctc

SEQ ID NO: 46 - RNA, 28 nt, synthetic construct
  source 1..28: mol_type = other RNA
cgctattgtgggtcgttacgtacttagc

SEQ ID NO: 47 - RNA, 59 nt, synthetic construct
  source 1..59: mol_type = other RNA
catcaccacagccaggatccgatgtcaacgattattatggatttatgtagttacacccg

SEQ ID NO: 48 - RNA, 53 nt, synthetic construct
  source 1..53: mol_type = other RNA
cattatgcggccgcaagcttttagcgcatgttgacaaaaataccattagtcac

SEQ ID NO: 49 - RNA, 55 nt, synthetic construct
  source 1..55: mol_type = other RNA
aaggagatataccatataccatgaacaatatgaacgtaattattgccgatgacca

SEQ ID NO: 50 - RNA, 51 nt, synthetic construct
  source 1..51: mol_type = other RNA
ccgagctcgaattcggatccttagtctttatctgccggacttaaggtcact

SEQ ID NO: 51 - RNA, 49 nt, synthetic construct
  source 1..49: mol_type = other RNA
aaggagatataccatataccatgaaaaacatcaatccaacgcagaccgc

SEQ ID NO: 52 - RNA, 54 nt, synthetic construct
  source 1..54: mol_type = other RNA
cgccgagctcgaattcggatccttaaccgcgccacgctttatagcggttaatca

SEQ ID NO: 53 - RNA, 44 nt, synthetic construct
  source 1..44: mol_type = other RNA
aaggagatataccatataccatggcaatccacaatcgtgcaggc

SEQ ID NO: 54 - RNA, 51 nt, synthetic construct
  source 1..51: mol_type = other RNA
cgccgagctcgaattcggatccttacgcgtttttcagaacttcgctaacaa

SEQ ID NO: 55 - RNA, 51 nt, synthetic construct
  source 1..51: mol_type = other RNA
aaggagatataccatataccatggctgccattaatacgaaagtcaaaaaag

SEQ ID NO: 56 - RNA, 53 nt, synthetic construct
  source 1..53: mol_type = other RNA
cgccgagctcgaattcggatccttacttcttaatgcccatctcttcttcaagc

SEQ ID NO: 57 - RNA, 46 nt, synthetic construct
  source 1..46: mol_type = other RNA
aaggagatataccatataccatgagagttctggttaccggtggtag

SEQ ID NO: 58 - RNA, 50 nt, synthetic construct
  source 1..50: mol_type = other RNA
cgccgagctcgaattcggatccttaatcgggatatccctgtggatggcgt

SEQ ID NO: 59 - RNA, 47 nt, synthetic construct
  source 1..47: mol_type = other RNA
aaggagatataccatataccatgaaaatcaccatttccggtactggc

SEQ ID NO: 60 - RNA, 48 nt, synthetic construct
  source 1..48: mol_type = other RNA
cgccgagctcgaattcggatccttagtcgctgccaaagagatcgcggg

SEQ ID NO: 61 - RNA, 50 nt, synthetic construct
  source 1..50: mol_type = other RNA
aaggagatataccatataccatgcaaaaactcattaactcagtgcaaaac

SEQ ID NO: 62 - RNA, 50 nt, synthetic construct
  source 1..50: mol_type = other RNA
cgccgagctcgaattcggatccttacagcttgttgtaaacacgcgctaaa

SEQ ID NO: 63 - RNA, 51 nt, synthetic construct
  source 1..51: mol_type = other RNA
aaggagatataccatataccatgaaaaaattaacctgctttaaagcctatg

SEQ ID NO: 64 - RNA, 46 nt, synthetic construct
  source 1..46: mol_type = other RNA
cgccgagctcgaattcggatccttactcgttcagcaacgtcagcag

SEQ ID NO: 65 - DNA, 45 bp, synthetic construct
  source 1..45: mol_type = other DNA
agaaggagatataccatataccatggcgcagtcgaaactctatcc

SEQ ID NO: 66 - RNA, 47 nt, synthetic construct
  source 1..47: mol_type = other RNA
cgccgagctcgaattcggatccttacacccgtccgtagcgatccgcg

SEQ ID NO: 67 - RNA, 45 nt, synthetic construct
  source 1..45: mol_type = other RNA
aaggagatataccatataccatgtcaaaagtcgctctcatcaccg

SEQ ID NO: 68 - RNA, 44 nt, synthetic construct
  source 1..44: mol_type = other RNA
cgccgagctcgaattcggatccttatgactccagcgcgatcgcc

SEQ ID NO: 69 - RNA, 48 nt, synthetic construct
  source 1..48: mol_type = other RNA
aaggagatataccatataccatgagtaaacaacgagtttttattgctg

SEQ ID NO: 70 - RNA, 43 nt, synthetic construct
  source 1..43: mol_type = other RNA
cgccgagctcgaattcggatccttacccccgaaagcggtcttg

SEQ ID NO: 71 - RNA, 20 nt, synthetic construct
  source 1..20: mol_type = other RNA
ctgctgctcggtattcaaag

SEQ ID NO: 72 - RNA, 25 nt, synthetic construct
  source 1..25: mol_type = other RNA
actagtattatacctaggactgagc

SEQ ID NO: 73 - RNA, 20 nt, synthetic construct
  source 1..20: mol_type = other RNA
tgtgtagatgagattgcacg

SEQ ID NO: 74 - RNA, 20 nt, synthetic construct
  source 1..20: mol_type = other RNA
acgtcgcgaagaagaaagcg

SEQ ID NO: 75 - RNA, 20 nt, synthetic construct
  source 1..20: mol_type = other RNA
ggtcaggcaagaaaccagcg